European Patent Specification EP 3 615 561 B1, published January 10, 2024. Title: Variants of Human BMP7 Protein. Applicant: Eli Lilly and Company. The sequence listing filed with the application follows.

SEQUENCE LISTING (21 sequences)

SEQ ID NO: 1 - protein, 431 aa, Homo sapiens
MHVRSLRAAAPHSFVALWAPLFLLRSALADFSLDNEVHSSFIHRRLRSQERREMQREILSILGLPHRPRPHLQGKHNSAPMFMLDLYNAMAVEEGGGPGGQGFSYPYKAVFSTQGPPLASLQDSHFLTDADMVMSFVNLVEHDKEFFHPRYHHREFRFDLSKIPEGEAVTAAEFRIYKDYIRERFDNETFRISVYQVLQEHLGRESDLFLLDSRTLWASEEGWLVFDITATSNHWVVNPRHNLGLQLSVETLDGQSINPKLAGLIGRHGPQNKQPFMVAFFKATEVHFRSIRSTGSKQRSQNRSKTPKNQEALRMANVAENSSSDQRQACKKHELYVSFRDLGWQDWIIAPEGYAAYYCEGECAFPLNSYMNATNHAIVQTLVHFINPETVPKPCCAPTQLNAISVLYFDDSSNVILKKYRNMVVRACGCH

SEQ ID NO: 2 - protein, 139 aa, Homo sapiens
STGSKQRSQNRSKTPKNQEALRMANVAENSSSDQRQACKKHELYVSFRDLGWQDWIIAPEGYAAYYCEGECAFPLNSYMNATNHAIVQTLVHFINPETVPKPCCAPTQLNAISVLYFDDSSNVILKKYRNMVVRACGCH

SEQ ID NO: 3 - protein, 139 aa, Artificial Sequence
  Synthetic construct
  MISC_FEATURE (33)..(33): Xaa at position 33 = D or M
  MISC_FEATURE (37)..(37): Xaa at position 37 = A or P
  MISC_FEATURE (60)..(60): Xaa at position 60 = E or Q
  MISC_FEATURE (65)..(65): Xaa at position 65 = Y, S, or G
  MISC_FEATURE (86)..(86): Xaa at position 86 = I, V, or L
  MISC_FEATURE (87)..(87): Xaa at position 87 = V or L
  MISC_FEATURE (89)..(89): Xaa at position 89 = T, S, or A
  MISC_FEATURE (91)..(91): Xaa at position 91 = V or M
  MISC_FEATURE (93)..(93): Xaa at position 93 = F or V
  MISC_FEATURE (94)..(94): Xaa at position 94 = I, F, or M
  MISC_FEATURE (110)..(110): Xaa at position 110 = N, A, S, or G
  MISC_FEATURE (114)..(114): Xaa at position 114 = V or M
  MISC_FEATURE (120)..(120): Xaa at position 120 = S or Q
  MISC_FEATURE (128)..(128): Xaa at position 128 = Y, F or W
  MISC_FEATURE (132)..(132): Xaa at position 132 = V, Q, or S
  MISC_FEATURE (134)..(134): Xaa at position 134 = R or K
STGSKQRSQNRSKTPKNQEALRMANVAENSSSXQRQXCKKHELYVSFRDLGWQDWIIAPXGYAAXYCEGECAFPLNSYMNATNHAXXQXLXHXXNPETVPKPCCAPTQLXAISXLYFDDXSNVILKKXRNMXVXACGCH

SEQ ID NO: 4 - protein, 139 aa, Artificial Sequence
  Synthetic construct
STGSKQRSQNRSKTPKNQEALRMANVAENSSSDQRQACKKHELYVSFRDLGWQDWIIAPEGYAAYYCEGECAFPLNSYMNATNHAIVQTLVHVINPETVPKPCCAPTQLGAISVLYFDDSSNVILKKYRNMVVRACGCH

SEQ ID NO: 5 - protein, 139 aa, Artificial Sequence
  Synthetic construct
STGSKQRSQNRSKTPKNQEALRMANVAENSSSDQRQACKKHELYVSFRDLGWQDWIIAPEGYAAGYCEGECAFPLNSYMNATNHALVQALVHFINPETVPKPCCAPTQLGAISVLYFDDSSNVILKKYRNMVVRACGCH

SEQ ID NO: 6 - protein, 139 aa, Artificial Sequence
  Synthetic construct
STGSKQRSQNRSKTPKNQEALRMANVAENSSSDQRQACKKHELYVSFRDLGWQDWIIAPEGYAAGYCEGECAFPLNSYMNATNHALVQTLVHFINPETVPKPCCAPTQLGAISVLYFDDSSNVILKKFRNMVVRACGCH

SEQ ID NO: 7 - protein, 139 aa, Artificial Sequence
  Synthetic construct
STGSKQRSQNRSKTPKNQEALRMANVAENSSSDQRQACKKHELYVSFRDLGWQDWIIAPEGYAAGYCEGECAFPLNSYMNATNHALVQTLVHFINPETVPKPCCAPTQLGAISVLYFDDSSNVILKKWRNMVVRACGCH

SEQ ID NO: 8 - protein, 139 aa, Artificial Sequence
  Synthetic construct
STGSKQRSQNRSKTPKNQEALRMANVAENSSSDQRQACKKHELYVSFRDLGWQDWIIAPEGYAAGYCEGECAFPLNSYMNATNHALVQTLVHVINPETVPKPCCAPTQLGAISVLYFDDSSNVILKKWRNMVVRACGCH

SEQ ID NO: 9 - protein, 139 aa, Artificial Sequence
  Synthetic construct
STGSKQRSQNRSKTPKNQEALRMANVAENSSSDQRQACKKHELYVSFRDLGWQDWIIAPEGYAAGYCEGECAFPLNSYMNATNHAIVQALVHFINPETVPKPCCAPTQLGAISVLYFDDSSNVILKKFRNMVVRACGCH

SEQ ID NO: 10 - protein, 139 aa, Artificial Sequence
  Synthetic construct
STGSKQRSQNRSKTPKNQEALRMANVAENSSSDQRQACKKHELYVSFRDLGWQDWIIAPEGYAAGYCEGECAFPLNSYMNATNHALVQTLVHFINPETVPKPCCAPTQLGAISVLYFDDSSNVILKKYRNMVVRACGCH

SEQ ID NO: 11 - protein, 139 aa, Artificial Sequence
  Synthetic construct
STGSKQRSQNRSKTPKNQEALRMANVAENSSSDQRQACKKHELYVSFRDLGWQDWIIAPEGYAAGYCEGECAFPLNSYMNATNHAIVQTLVHFINPETVPKPCCAPTQLNAISMLYFDDSSNVILKKYRNMVVRACGCH

SEQ ID NO: 12 - protein, 402 aa, Artificial Sequence
  Synthetic construct
DFSLDNEVHSSFIHRRLRSQERREMQREILSILGLPHRPRPHLQGKHNSAPMFMLDLYNAMAVEEGGGPGGQGFSYPYKAVFSTQGPPLASLQDSHFLTDADMVMSFVNLVEHDKEFFHPRYHHREFRFDLSKIPEGEAVTAAEFRIYKDYIRERFDNETFRISVYQVLQEHLGRESDLFLLDSRTLWASEEGWLVFDITATSNHWVVNPRHNLGLQLSVETLDGQSINPKLAGLIGRHGPQNKQPFMVAFFKATEVHFRSIRSTGSKQRSQNRSKTPKNQEALRMANVAENSSSDQRQACKKHELYVSFRDLGWQDWIIAPEGYAAYYCEGECAFPLNSYMNATNHAIVQTLVHVINPETVPKPCCAPTQLGAISVLYFDDSSNVILKKYRNMVVRACGCH

SEQ ID NO: 13 - protein, 402 aa, Artificial Sequence
  Synthetic construct
DFSLDNEVHSSFIHRRLRSQERREMQREILSILGLPHRPRPHLQGKHNSAPMFMLDLYNAMAVEEGGGPGGQGFSYPYKAVFSTQGPPLASLQDSHFLTDADMVMSFVNLVEHDKEFFHPRYHHREFRFDLSKIPEGEAVTAAEFRIYKDYIRERFDNETFRISVYQVLQEHLGRESDLFLLDSRTLWASEEGWLVFDITATSNHWVVNPRHNLGLQLSVETLDGQSINPKLAGLIGRHGPQNKQPFMVAFFKATEVHFRSIRSTGSKQRSQNRSKTPKNQEALRMANVAENSSSDQRQACKKHELYVSFRDLGWQDWIIAPEGYAAGYCEGECAFPLNSYMNATNHALVQALVHFINPETVPKPCCAPTQLGAISVLYFDDSSNVILKKYRNMVVRACGCH

SEQ ID NO: 14 - protein, 402 aa, Artificial Sequence
  Synthetic construct
DFSLDNEVHSSFIHRRLRSQERREMQREILSILGLPHRPRPHLQGKHNSAPMFMLDLYNAMAVEEGGGPGGQGFSYPYKAVFSTQGPPLASLQDSHFLTDADMVMSFVNLVEHDKEFFHPRYHHREFRFDLSKIPEGEAVTAAEFRIYKDYIRERFDNETFRISVYQVLQEHLGRESDLFLLDSRTLWASEEGWLVFDITATSNHWVVNPRHNLGLQLSVETLDGQSINPKLAGLIGRHGPQNKQPFMVAFFKATEVHFRSIRSTGSKQRSQNRSKTPKNQEALRMANVAENSSSDQRQACKKHELYVSFRDLGWQDWIIAPEGYAAGYCEGECAFPLNSYMNATNHALVQTLVHFINPETVPKPCCAPTQLGAISVLYFDDSSNVILKKFRNMVVRACGCH

SEQ ID NO: 15 - protein, 402 aa, Artificial Sequence
  Synthetic construct
DFSLDNEVHSSFIHRRLRSQERREMQREILSILGLPHRPRPHLQGKHNSAPMFMLDLYNAMAVEEGGGPGGQGFSYPYKAVFSTQGPPLASLQDSHFLTDADMVMSFVNLVEHDKEFFHPRYHHREFRFDLSKIPEGEAVTAAEFRIYKDYIRERFDNETFRISVYQVLQEHLGRESDLFLLDSRTLWASEEGWLVFDITATSNHWVVNPRHNLGLQLSVETLDGQSINPKLAGLIGRHGPQNKQPFMVAFFKATEVHFRSIRSTGSKQRSQNRSKTPKNQEALRMANVAENSSSDQRQACKKHELYVSFRDLGWQDWIIAPEGYAAGYCEGECAFPLNSYMNATNHALVQTLVHFINPETVPKPCCAPTQLGAISVLYFDDSSNVILKKWRNMVVRACGCH

SEQ ID NO: 16 - protein, 402 aa, Artificial Sequence
  Synthetic construct
DFSLDNEVHSSFIHRRLRSQERREMQREILSILGLPHRPRPHLQGKHNSAPMFMLDLYNAMAVEEGGGPGGQGFSYPYKAVFSTQGPPLASLQDSHFLTDADMVMSFVNLVEHDKEFFHPRYHHREFRFDLSKIPEGEAVTAAEFRIYKDYIRERFDNETFRISVYQVLQEHLGRESDLFLLDSRTLWASEEGWLVFDITATSNHWVVNPRHNLGLQLSVETLDGQSINPKLAGLIGRHGPQNKQPFMVAFFKATEVHFRSIRSTGSKQRSQNRSKTPKNQEALRMANVAENSSSDQRQACKKHELYVSFRDLGWQDWIIAPEGYAAGYCEGECAFPLNSYMNATNHALVQTLVHVINPETVPKPCCAPTQLGAISVLYFDDSSNVILKKWRNMVVRACGCH

SEQ ID NO: 17 - protein, 139 aa, Artificial Sequence
  Synthetic construct
  MISC_FEATURE (33)..(33): Xaa at position 33 = D or M
  MISC_FEATURE (37)..(37): Xaa at position 37 = A or P
  MISC_FEATURE (60)..(60): Xaa at position 60 = E or Q
  MISC_FEATURE (65)..(65): Xaa at position 65 = Y, S, or G
  MISC_FEATURE (86)..(86): Xaa at position 86 = I, V or L
  misc_feature (89)..(89): Xaa can be any naturally occurring amino acid
  MISC_FEATURE (91)..(91): Xaa at position 91 = V or M
  MISC_FEATURE (93)..(93): Xaa at 93 = F or V
  MISC_FEATURE (94)..(94): Xaa at 94 = I, F or M
  MISC_FEATURE (110)..(110): Xaa at position 110 = N, A, S or G
  MISC_FEATURE (114)..(114): Xaa at position 114 = V or M
  MISC_FEATURE (128)..(128): Xaa at position 128 = Y, F or W
STGSKQRSQNRSKTPKNQEALRMANVAENSSSXQRQXCKKHELYVSFRDLGWQDWIIAPXGYAAXYCEGECAFPLNSYMNATNHAXVQXLXHXXNPETVPKPCCAPTQLXAISXLYFDDSSNVILKKXRNMVVRACGCH

SEQ ID NO: 18 - protein, 257 aa, Artificial Sequence
  Synthetic construct
DFSLDNEVHSSFIHRRLRSQERREMQREILSILGLPHRPRPHLQGKHNSAPMFMLDLYNAMAVEEGGGPGGQGFSYPYKAVFSTQGPPLASLQDSHFLTDADMVMSFVNLVEHDKEFFHPRYHHREFRFDLSKIPEGEAVTAAEFRIYKDYIRERFDNETFRISVYQVLQSDLFLLDSRTLWASEEGWLVFDITATSNHWVVNPRHNLGLQLSVETLDGQSINPKLAGLIGRHGPQNKQPFMVAFFKATEVHFRSIR

SEQ ID NO: 19 - DNA, 1293 bp, Artificial Sequence
  Synthetic construct
atgcacgtgcgcagcctgcgcgccgccgccccccacagcttcgtggccctgtgggcccccctgttcctgctgcgcagcgccctggccgacttcagcctggacaacgaggtgcacagcagcttcatccaccgccgcctgcgcagccaggagcgccgcgagatgcagcgcgagatcctgagcatcctgggcctgccccaccgcccccgcccccacctgcagggcaagcacaacagcgcccccatgttcatgctggacctgtacaacgccatggccgtggaggagggcggcggccccggcggccagggcttcagctacccctacaaggccgtgttcagcacccagggcccccccctggccagcctgcaggacagccacttcctgaccgacgccgacatggtgatgagcttcgtgaacctggtggagcacgacaaggagttcttccacccccgctaccaccaccgcgagttccgcttcgacctgagcaagatccccgagggcgaggccgtgaccgccgccgagttccgcatctacaaggactacatccgcgagcgcttcgacaacgagaccttccgcatcagcgtgtaccaggtgctgcaggagcacctgggccgcgagagcgacctgttcctgctggacagccgcaccctgtgggccagcgaggagggctggctggtgttcgacatcaccgccaccagcaaccactgggtggtgaacccccgccacaacctgggcctgcagctgagcgtggagaccctggacggccagagcatcaaccccaagctggccggcctgatcggccgccacggcccccagaacaagcagcccttcatggtggccttcttcaaggccaccgaggtgcacttccgcagcatccgcagcaccggcagcaagcagcgcagccagaaccgcagcaagacccccaagaaccaggaggccctgcgcatggccaacgtggccgagaacagcagcagcgaccagcgccaggcctgcaagaagcacgagctgtacgtgagcttccgcgacctgggctggcaggactggatcatcgcccctgagggctacgccgccggctactgcgagggcgagtgcgccttccccctgaacagctacatgaacgccaccaaccacgccctggtgcagaccctggtgcacttcatcaaccccgagaccgtgcccaagccctgctgcgcccccacccagctgggcgccatcagcgtgctgtacttcgacgacagcagcaacgtgatcctgaagaagtggcgcaacatggtggtgcgcgcctgcggctgccac

SEQ ID NO: 20 - DNA, 1293 bp, Artificial Sequence
  Synthetic construct
atgcacgtgcgcagcctgcgcgccgccgccccccacagcttcgtggccctgtgggcccccctgttcctgctgcgcagcgccctggccgacttcagcctggacaacgaggtgcacagcagcttcatccaccgccgcctgcgcagccaggagcgccgcgagatgcagcgcgagatcctgagcatcctgggcctgccccaccgcccccgcccccacctgcagggcaagcacaacagcgcccccatgttcatgctggacctgtacaacgccatggccgtggaggagggcggcggccccggcggccagggcttcagctacccctacaaggccgtgttcagcacccagggcccccccctggccagcctgcaggacagccacttcctgaccgacgccgacatggtgatgagcttcgtgaacctggtggagcacgacaaggagttcttccacccccgctaccaccaccgcgagttccgcttcgacctgagcaagatccccgagggcgaggccgtgaccgccgccgagttccgcatctacaaggactacatccgcgagcgcttcgacaacgagaccttccgcatcagcgtgtaccaggtgctgcaggagcacctgggccgcgagagcgacctgttcctgctggacagccgcaccctgtgggccagcgaggagggctggctggtgttcgacatcaccgccaccagcaaccactgggtggtgaacccccgccacaacctgggcctgcagctgagcgtggagaccctggacggccagagcatcaaccccaagctggccggcctgatcggccgccacggcccccagaacaagcagcccttcatggtggccttcttcaaggccaccgaggtgcacttccgcagcatccgcagcaccggcagcaagcagcgcagccagaaccgcagcaagacccccaagaaccaggaggccctgcgcatggccaacgtggccgagaacagcagcagcgaccagcgccaggcctgcaagaagcacgagctgtacgtgagcttccgcgacctgggctggcaggactggatcatcgcccctgagggctacgccgccggctactgcgagggcgagtgcgccttccccctgaacagctacatgaacgccaccaaccacgccctggtgcagaccctggtgcacgtgatcaaccccgagaccgtgcccaagccctgctgcgcccccacccagctgggcgccatcagcgtgctgtacttcgacgacagcagcaacgtgatcctgaagaagtggcgcaacatggtggtgcgcgcctgcggctgccac

SEQ ID NO: 21 - protein, 402 aa, Homo sapiens
DFSLDNEVHSSFIHRRLRSQERREMQREILSILGLPHRPRPHLQGKHNSAPMFMLDLYNAMAVEEGGGPGGQGFSYPYKAVFSTQGPPLASLQDSHFLTDADMVMSFVNLVEHDKEFFHPRYHHREFRFDLSKIPEGEAVTAAEFRIYKDYIRERFDNETFRISVYQVLQEHLGRESDLFLLDSRTLWASEEGWLVFDITATSNHWVVNPRHNLGLQLSVETLDGQSINPKLAGLIGRHGPQNKQPFMVAFFKATEVHFRSIRSTGSKQRSQNRSKTPKNQEALRMANVAENSSSDQRQACKKHELYVSFRDLGWQDWIIAPEGYAAYYCEGECAFPLNSYMNATNHAIVQTLVHFINPETVPKPCCAPTQLNAISVLYFDDSSNVILKKYRNMVVRACGCH